European Patent Application EP 4 234 578 A1, published August 30, 2023. Title: The immunotherapeutic nanocage displaying PD-L1 binding peptide 1 and use in anti-cancer immunotherapeutic agent thereof. Applicant: KYUNGPOOK NATIONAL UNIVERSITY INDUSTRY-ACADEMIC COOPERATION FOUNDATION. The sequence listing filed with the application follows.

SEQUENCE LISTING (4 sequences)

SEQ ID NO: 1 - protein, 161 aa, Human
MTTASTSQVRQNYHQDSEAAINRQINLELYASYVYLSMSYYFDRDDVALKNFAKYFLHQSHEEREHAEKLMKLQNQRGGRIFLQDIKKPDCDDWESGLNAMECALHLEKNVNQSLLELHKLATDKNDPHLCDFIETHYLNEQVKAIKELGDHVTNLRKMGA

SEQ ID NO: 2 - protein, 9 aa, Artificial Sequence
  PD-L1 binding peptide 1
CLQKTPKQC

SEQ ID NO: 3 - protein, 2 aa, Artificial Sequence
  linker
GG

SEQ ID NO: 4 - protein, 10 aa, Artificial Sequence
  linker
GGGSGGGGSG